European Patent Application EP 4 119 658 A1, published January 18, 2023. Title: Phytase variants. Applicant: AB Enzymes. The sequence listing filed with the application follows.

SEQUENCE LISTING (2 sequences)

SEQ ID NO: 1 - protein, 410 aa, Artificial Sequence
  variant
QSEPELKLESVVIVSRHGVRAPTKFTQLMQDVTPDAWPTWPVKLGELTPRGGELIAYLGHYWRQRLVADGLLPKEGCPQSGQVAIIADVDERTRKTGEAFAAGLAPDCAITVHHQADTSSPDPLFNPLKTGVCQLDVANVRRAILERAGGSIADFTRHYQTAFRELERVLNFPQSNLCLKREKQDESCSLTQALPSELKVSADDVSLTGAVSLASMLTEIFLLQQAQGMPEPGWGRITDSHQWNTLLSLHNAYFDLLQRTPEVARSRATPLLDLIKTALTPHPPQKQAYGVTLPTSVLFIAGHDTNLANLGGALELNWTLPGQPDNYPPGGELVFERWRRLSDNSQWIQVSLVFQTLQQMRDKTPLSLNTPPGEVKLTLAGCEERNAQGMCSLAGFTQIVNEARIPACSL

SEQ ID NO: 2 - protein, 410 aa, Artificial Sequence
  variant
QSEPELKLESVVIVSRHGVRAPTKFTQLMQDVTPDAWPTWPVKLGELTPRGGELIAYLGHYWRQRLVADGLLPKEGCPQSGQVAIIADVDERTRKTGEAFAAGLAPDCAITVHHQADTSSPDPLFNPLKTGVCQLDVANVRRAILERAGGSIADFTRHYQTAFRELERVLNFPQSNLCLKREKQDESCSLTQALPSELKVSADDVSLTGAWSLASMLTEIFLLQQAQGMPEPGWGRITDSHQWNTLLSLHNAVFDLLQRTPEVARSRATPLLDLIKTALTPHPPQKQAYGVTLPTSVLFIAGHDTNLANLGGALELNWTLPGQPDNYPPGGELVFERWRRLSDNSQWIQVSLVFQTLQQMRDKTPLSLNTPPGEVKLTLAGCEERNAQGMCSLAGFTQIVNEARIPACSL